European Patent Application EP 4 272 821 A2, published November 8, 2023. Title: TREATMENT OF INFLAMMATORY DISEASES WITH INHIBITORS OF C5A ACTIVITY. Applicant: InflaRx GmbH. The sequence listing filed with the application follows.

SEQUENCE LISTING (34 sequences)

SEQ ID NO: 1 - protein, 74 aa, Homo sapiens
TLQKKIEEIAAKYKHSVVKKCCYDGACVNNDETCEQRAARISLGPRCIKAFTECCVVASQLRANISHKDMQLGR

SEQ ID NO: 2 - protein, 9 aa, Homo sapiens
NDETCEQRA

SEQ ID NO: 3 - protein, 7 aa, Homo sapiens
SHKDMQL

SEQ ID NO: 4 - protein, 7 aa, Homo sapiens
DETCEQR

SEQ ID NO: 5 - protein, 5 aa, Homo sapiens
HKDMQ

SEQ ID NO: 6 - protein, 13 aa, synthetic construct
  REGION 1..13: note = IFX-1 CDR3 heavy chain
CARGNDGYYGFAY

SEQ ID NO: 7 - protein, 15 aa, synthetic construct
  REGION 1..15: note = INab708 CDR3 heavy chain
CTRRGLYDGSSYFAY

SEQ ID NO: 8 - protein, 10 aa, synthetic construct
  REGION 1..10: note = IFX-1 CDR3 light chain
CQQSNEDPYT

SEQ ID NO: 9 - protein, 10 aa, synthetic construct
  REGION 1..10: note = INab708 CDR3 light chain
CQQNNEDPLT

SEQ ID NO: 10 - protein, 12 aa, synthetic construct
  REGION 1..12: note = IFX-1 CDR2 heavy chain
IDPSDSESRLDQ

SEQ ID NO: 11 - protein, 12 aa, synthetic construct
  REGION 1..12: note = INab708 CDR2 heavy chain
ILPGSGSTNYNE

SEQ ID NO: 12 - protein, 7 aa, synthetic construct
  REGION 1..7: note = IFX-1 CDR2 light chain
IYAASNL

SEQ ID NO: 13 - protein, 7 aa, synthetic construct
  REGION 1..7: note = INab708 CDR2 light chain
IYAASNL

SEQ ID NO: 14 - protein, 14 aa, synthetic construct
  REGION 1..14: note = IFX-1 CDR1 heavy chain
CKASGYSFTTFWMD

SEQ ID NO: 15 - protein, 14 aa, synthetic construct
  REGION 1..14: note = INab708 CDR1 heavy chain
CKATGNTFSGYWIE

SEQ ID NO: 16 - protein, 16 aa, synthetic construct
  REGION 1..16: note = IFX-1 CDR1 light chain
CKASQSVDYDGDSYMK

SEQ ID NO: 17 - protein, 16 aa, synthetic construct
  REGION 1..16: note = INab708 CDR1 light chain
CKASQSVDYDGDSYMN

SEQ ID NO: 18 - protein, 21 aa, synthetic construct
  REGION 1..21: note = IFX-1 FR1 heavy chain
QVQLQQSGPQLVRPGTSVKIS

SEQ ID NO: 19 - protein, 15 aa, synthetic construct
  REGION 1..15: note = IFX-1 FR2 heavy chain
WVKQRPGQGLEWIGR

SEQ ID NO: 20 - protein, 33 aa, synthetic construct
  REGION 1..33: note = IFX-1 FR3 heavy chain
RFKDRATLTVDKSSSTVYMQLSSPTSEDSAVYY

SEQ ID NO: 21 - protein, 11 aa, synthetic construct
  REGION 1..11: note = IFX-1 FR4 heavy chain
WGQGTLVTVSS

SEQ ID NO: 22 - protein, 22 aa, synthetic construct
  REGION 1..22: note = IFX-1 FR1 light chain
DIVLTQSPASLAVSLGQRATIS

SEQ ID NO: 23 - protein, 13 aa, synthetic construct
  REGION 1..13: note = IFX-1 FR2 light chain
WYQQKPGQPPKLL

SEQ ID NO: 24 - protein, 33 aa, synthetic construct
  REGION 1..33: note = IFX-1 FR3 light chain
QSGIPARFSGSGSGTDFTLNIHPVEEEDAATYY

SEQ ID NO: 25 - protein, 10 aa, synthetic construct
  REGION 1..10: note = IFX-1 FR4 light chain
FGGGTKLEIK

SEQ ID NO: 26 - protein, 20 aa, synthetic construct
  REGION 1..20: note = INab708 FR1 heavy chain
VQLLESGAELMKPGASVKIS

SEQ ID NO: 27 - protein, 15 aa, synthetic construct
  REGION 1..15: note = INab708 FR2 heavy chain
WVKQRPGHGLEWIGE

SEQ ID NO: 28 - protein, 33 aa, synthetic construct
  REGION 1..33: note = INab708 FR3 heavy chain
KFKGKATLTADTSSNTAYMQLSSLTSEDSAVYY

SEQ ID NO: 29 - protein, 11 aa, synthetic construct
  REGION 1..11: note = INab708 FR4 heavy chain
WGQGTLVTVSA

SEQ ID NO: 30 - protein, 22 aa, synthetic construct
  REGION 1..22: note = INab708 FR1 light chain
DIVLTQSPASLAVSLGQRATIS

SEQ ID NO: 31 - protein, 13 aa, synthetic construct
  REGION 1..13: note = INab708 FR2 light chain
WYQQKPGQPPKLL

SEQ ID NO: 32 - protein, 33 aa, synthetic construct
  REGION 1..33: note = INab708 FR3 light chain
GSGIPARFSGSGSGTDFTLNIHPVEEEVAATYY

SEQ ID NO: 33 - protein, 10 aa, synthetic construct
  REGION 1..10: note = INab708 FR4 light chain
FGAGTLLELK

SEQ ID NO: 34 - RNA, 40 nt, synthetic construct
  misc_feature 1..40: note = pegylated mixed L-RNA/DNA-aptamer NOX-D21
  misc_feature 1: note = substituted by 40 kDaPEG-aminohexyl-
  misc_feature 7: note = desoxy uridine
  misc_feature 28: note = desoxy uridine
  misc_feature 38: note = desoxy cytidine
  source 1..40: mol_type = other RNA
gcgatgtggtggtgaagggttgttgggtgtcgacgcacgc